European Patent Application EP 4 772 632 A1, published July 8, 2026. Title: gRNA及其生物合成方法. Applicant: 吉林凯莱英医药化学有限公司. The sequence listing filed with the application follows.

SEQUENCE LISTING (52 sequences)

SEQ ID NO: 1 - protein, 374 aa, Bacteriophage T4
MQELFNNLMELCKDSQRKFFYSDDVSASGRTYRIFSYNYASYSDWLLPDALECRGIMFEMDGEKPVRIASRPMEKFFNLNENPFTMNIDLNDVDYILTKEDGSLVSTYLDGDEILFKSKGSIKSEQALMANGILMNINHHRLRDRLKELAEDGFTANFEFVAPTNRIVLAYQEMKIILLNVRENETGEYISYDDIYKDATLRPYLVERYEIDSPKWIEEAKNAENIEGYVAVMKDGSHFKIKSDWYVSLHSTKSSLDNPEKLFKTIIDGASDDLKAMYADDEYSYRKIEAFETTYLKYLDRALFLVLDCHNKHCGKDRKTYAMEAQGVAKGAGMDHLFGIIMSLYQGYDSQEKVMCEIEQNFLKNYKKFIPEGY

SEQ ID NO: 2 - protein, 335 aa, Salmonella phage STP4-a
MFKKYSSLENHYNNKFISKIRFEGKDGGLWVAREKIHGTNFSIIVSKDSVSACKRSGPILPSESFYGHEIILKNYDESIKTIQRCMNANELGSVSSYQIFGEFAGQGIQKEVDYGEKDFYVFDILVNTQNGNVLYMDDMMMTSFCNEFGFKMAPFIGCGSFDELIQLPNNFTSVIKAYNEAAKDDLKEVNLCVFDPLVTDDNVAEGYVLKPVYPDFFNNGTRIAIKSKNSRFTEKKKSDKPIKPKAVLTSNDSTVLANLCEYSTWNRVSNVISHIGEVKAKDFGKVMGLTIQDIFIEAKREGVDIVHADNPDLVKRELQTVVSNTIREKWLEIVS

SEQ ID NO: 3 - protein, 334 aa, Bacteriophage T4
MFKKYSSLENHYNSKFIEKLYSLGLTGGEWVAREKIHGTNFSLIIERDKVTCAKRTGPILPAEDFFGYEIILKNYADSIKAVQDIMETSAVVSYQVFGEFAGPGIQKNVDYCDKDFYVFDIIVTTESGDVTYVDDYMMESFCNTFKFKMAPLLGRGKFEELIKLPNDLDSVVQDYNFTVDHAGLVDANKCVWNAEAKGEVFTAEGYVLKPCYPSWLRNGNRVAIKCKNSKFSEKKKSDKPIKAKVELSEADNKLVGILACYVTLNRVNNVISKIGEIGPKDFGKVMGLTVQDILEETSREGITLTQADNPSLIKKELVKMVQDVLRPAWIELVS

SEQ ID NO: 4 - protein, 335 aa, Vibrio phage KVP40
MSFVKYTSLENSYRQAFVDKCDMLGVREWVALEKIHGANFSFIVEFKPNEAQDGAEFTVTPAKRTSTIGANVMGDYDFYGCTSVVEAHTAKMEAISNWLWARGIINVGETIIVYGELAGKGVQKEVNYGDKDFWAYDILLPETGKFLDWDVVLEACEFAKVKTTHEIARGTLDELLRIDPLFRSFHTPADVDGDNVAEGFVVKQLRNEKRLHNGSRAILKVKNDKFKEKKNKAGKTPRAAVVLTEEQEKLHAAFSCYLTENRLRNVLSKLETVTQKQFGMISGLFIKDAKDEFERDELNETAIARDDWDVIKRSLTNIANEILRKNWLDILDGNF

SEQ ID NO: 5 - protein, 379 aa, Pyrococcus abyssi
MVSSVYKEILVKLGLTEDRIETLEMKGGIIEDEFDGIRYVRFKDSAGKLRRGTVVIDEEYVIPGFPHIKRIINLRSGIRRIFKRGEFYVEEKVDGYNVRVVMYKGKMLGITRGGFICPFTTERIPDFVPQEFFKDNPNLILVGEMAGPESPYLVEGPPYVKEDIQFFLFDVQEIKTGRSLPVEERLKIAEEYGINHVEVFGKYTKDDVDELYQLIERLSKEGREGIIMKSPDMKKIVKYVTPYANINDIKIGARVFYELPPGYFTSRISRLAFYLAEKRIKGEEFERVAKELGSALLQPFVESIFDVEQEEDIHELFKVRVKRIETAYKMVTHFEKLGLKIEIVDIEEIKDGWRITFKRLYPDATNEIRELIGGKAFVD

SEQ ID NO: 6 - protein, 327 aa, Vibrio phage nt-1
MSFVKYTSLENSYRQAFVDKCDMLGVRDWVALEKIHGANFSFIVEFDGGYTVTPAKRTSIIGATATGDYDFYGCTSVVEAHKEKVELVANFLWLNEYINLYEPIIIYGELAGKGIQKEVNYGDKDFWAFDIFLPQREEFVDWDTCVAAFTNAEIKYTKELARGTLDELLRIDPLFKSLHTPAEHEGDNVAEGFVVKQLHSEKRLQSGSRAILKVKNEKFKEKKKKEGKTPTKLVLTPEQEKLHAEFSCYLTENRLKNVLSKLGTVNQKQFGMISGLFVKDAKDEFERDELNEVAIDRDDWNAIRRSLTNIANEILRKNWLNILDGNF

SEQ ID NO: 7 - protein, 374 aa, Shigella phage Sf22
MQELFNNLMELCKDSQRKFFYSDDVSASGRTYRIFSYNYASYSDWLLPDALECRGIMFEMDGEKPVRIASRPMEKFFNLNENPFTMNIDLNDVDYILTKEDGSLVSTYLDGDEILFKSKGSIKSEQALMANGILMNINHHQLRDRLKELAEDGFTANFEFVAPTNRIVLAYQEMKIILLNIRENETGEYISYDDIYKDAALRPYLVERFEVDSPKWIEEAKNAENIEGYVAVMKDGSHFKIKSDWYVSLHSTKSSLDNPEKLFKTIIDGASDDLKAMYADDEYSYRKIEAFETTYLKYLDRALFLVLDCHNKHCGKDRKTYAMEAQGVAKGAGMEHLFGIIMSLYQGYDSQEKVMCEIEQNFLKNYKKFIPEGY

SEQ ID NO: 8 - protein, 381 aa, Vibrio phage VH7D
MNVQELYKNLMSLADDAEGKFFFADHLSPLGEKFRVFSYHIASYSDWLLPGALEARGIMFQLDDNDEMIRIVSRPMEKFFNLNENPFTMELDLTTTVQLMDKADGSLISTYLSGENFALKSKTSIFSEQAVAANRYIKKPENRDLWEFCDDCTQAGLTVNMEWCAPNNRIVLEYPEAKLVILNIRDNETGDYVSFDDIPQSALMRVKQWLVDEYDPATAHEPDFVEKLRDTKGIEGMILRLANGQSVKIKTQWYVDLHSQKDSVNVPKKLVTTILNGNHDDLYALFADDKPTIERIREFDSHVTKTLTNSFNAVRQFYARNRHLARKDYAIAGQKVLKPWEFGVAMIAYQKQTVEGVYESLVTAYLKRPELAIPEKYLNGV

SEQ ID NO: 9 - protein, 335 aa, Escherichia phage dhaeg
MFKKYSSLENHYNSKFIEKLRTNGLTGGEWVAREKIHGTNFSLIIERDAVTCAKRTGPILPAEDFYGYEIVLKNYADSIKSIQDIMETSAAVSYQVFGEFAGTGIQKNVDYGDKDFYVFDIIVTTESGDVTYVDDYMMESFCKTFKFKMAPLLGRGKFEDLIKLPNDLDSVLPDYNFTVDNVGLAEANAHVWNAEAKGEVFTAEGYVLKPCYPLWLPNGNRVAIKCKNSKFSEKKKTDKPIKVAVVLSQDDLDLLQQFTDYVTVNRINNVISKIGEVSPKDFGKVMGLTVQDILEEAAREELELTDAENPVEVKKQLIECVKDTLRAVWIELVSK

SEQ ID NO: 10 - protein, 339 aa, Klebsiella phage KP27
MFKKYSSLTNHYEGKFINGVIMNGLTGGVWVAREKIHGANFSFITDDGITVTPAKRTDVVKPAEDFYGCSAVVAKYSPGIRKMWETLKKTGTYDDLVIQVYGEFAGRGVQKDVDYGEKDFYVFDIRVNGEFLPDNLCSLISRSHGLKMAPLLGYGTFEEIKELPITFESVVNKANSGIGSDNTVYGEFVYPIMDVEEGNIAEGFVMKPVSPAFMPNGERVAIKCKTTKFTEKKAKKATRFNAPVSLSEKDKNQLDEFVCYLTENRVKNVLSKLDLASITAKDFGRIMGLTVQDAIEEISRNHGPFLEQFEDPAMAKKLFVTEAQNMIRPVWGKILNHEF

SEQ ID NO: 11 - protein, 381 aa, Vibrio phage V05
MTTQELYNHLMTLTDDAEGKFFFADHISPLGEKLRVFSYHIASYSDWLLPGALEARGIMFQLDEQDKMVRIVSRPMEKFFNLNENPFTMDLDLTTTVQLMDKADGSLISTYLTGENFALKSKTSIFSEQAVAANRYIKLPENRDLWEFCDDLTQAGCTVNMEWCAPNNRIVLEYPEAKLVILNIRDNETGDYVSFDDIPLPALMRVKKWLVDEYDPETAHADDFVEKLRATKGIEGMILRLANGQSVKIKTQWYVDLHSQKDSVNVPKKLVTTILNNNHDDLYALFADDKPTIDRIREFDSHVSKTVSASFHAVSQFYVKNRHMSRKDYAIAGQKTLKPWEFGVAMIAYQNQTVEGVYEALVGAYLKRPELLIPEKYLNEA

SEQ ID NO: 12 - protein, 334 aa, Escherichia phage AR1
MFKKYSSLENHYNSKFIEKLYSLGLTGGEWVAREKIHGTNFSLIIERDKVTCAKRTGPILPAEDFFGYEIILKNYADSIKAVQDIMETSAVVSYQVFGEFAGPGIQKNVDYGDKDFYVFDIIVTTESGDMTYVDDYMMESFCNTFKFKMAPLLGRGKFEELIKLPNDLDSVVQDYNFTVDHAGLVDANKCVWNAEAKGEVFTAEGYVLKPCYPSWLPNRNRVAIKCKNSKFSEKKKSDKPIKAKVELSEADNKLVGILACYVTLNRVNNVISKIGEIGPKDFGKVMGLTVQDILEETSREGITLTQADNPSLIKKELVKMVQDVLRPAWIELVS

SEQ ID NO: 13 - protein, 438 aa, Bacteriophage RM378
MESMNVKYPVEYLIEHLNSFESPEVAVESLRKEGIMCKNRGDLYMFKYHLGCKFDKIYHLACRGAILRKTDSGWKVLSYPFDKFFNWGEELQPEIVNYYQTLRYASPLNEKRKAGFMFKLPMKLVEKLDGTCVVLYYDEGWKIHTLGSIDANGSIVKNGMVTTHMDKTYRELFWETFEKKYPPYLLYHLNSSYCYIFEMVHPDARVVVPYEEPNIILIGVRSVDPEKGYFEVGPSEEAVRIFNESGGKINLKLPAVLSQEQNYTLFRANRLQELFEEVTPLFKSLRDGYEVVYEGFVAVQEIAPRVYYRTKIKHPVYLELHRIKTTITPEKLADLFLENKLDDFVLTPDEQETVMKLKEIYTDMRNQLESSFDTIYKEISEQVSPEENPGEFRKRFALRLMDYHDKSWFFARLDGDEEKMQKSEKKLLTERIEKGLFK

SEQ ID NO: 14 - protein, 376 aa, Citrobacter phage CkP1
MKKLFKNLMALCDEADESKFFYRDDISPSGLKYRIFSYNYASYSDWIRPDALECRGIMFEMIDDKPVRIASRPMEKFFNLNETPFTMNLDLSKAKYMLDKADGSLVSTFLDGNILKFKSKSSIKSEQSYFSTAMLTESRHEALLARLLDLASDGFTANFEYVSPDNRIVLPYQEKQLILLNIRDNDTGEYVDYEDIFKDGVLRQYLVQRHEITDSNFVEDIRKLTDIEGFVFVMEDGLRFKLKTDWYCALHHTKDSITNNERLFESIVNNASDDLKAMFAGDEFAVNKINKFEENYLKYLGESLHLINTTYHELRGRDRKDYAIESQNRANKSGLGFLFSIIMKMYNGGMDHDTRVKNLSELFMKNYKQFVPKEFI

SEQ ID NO: 15 - protein, 374 aa, Escherichia phage JN02
MEKLYYNLLSLCKSSSDRKFFYSDDVSPIGKKYRIFSYNFASYSDWLLPDALECRGIMFEMDGETPVRIASRPMEKFFNLNENPFTLSINLDDVKYLMTKEDGSLVSTYLDGGTVRFKSKGSIKSDQAVSATSILLDIDHKNLADRLLELCNDGFTANFEYVAPTNKIVLTYPEKRLILLNIRDNNTGEYIEYDDIYLDPVFRKYLVDRFEVPEGDWTSDVKSSTNIEGYVAVMKDGSHFKLKTDWYVALHTTRDSISSPEKLFLAIVNGASDDLKAMYADDEFSFKKVELFEKAYLDFLDRSFYICLDTYDKHKGKDRKTYAIEAQAVCKGAQTPWLFGIIMNLYQGGSKEQMMTALESVFIKNHKNFIPEGY

SEQ ID NO: 16 - protein, 383 aa, Klebsiella phage KP179
MLELYKNLMNLCESSEVAKFFYKDFTGPMDGKFRVFSYHYASYSEWLKPDALECRGIMFEMDGDTPIRIASRPMEKFFNLNENPLTMGIDISDVEYIMDKADGSLVSSYVDDGYLYLKSKTSLYSDQARQASALLNSEEYSSLHQVILELTLDGYTVNMEFVSPNNRVVLAYQEPQLFVLNVRNNTTGEYIKYDDLYANAKIRPYLINAYGISDPTTWVEGVRELEGVEGYIAVLNTGQRFKVKTEWYSALHHTKDSITSNERLFASVVSANSDDLRSLFAGDEYAIKKISAFEQAYLDYLGKSLELCQSFYDEYRGRARKDYAIAAQKATVNQRHLFGVIMNMYEGTVDVDKLLKDLERVFLKYWAGYVPKEYEKEIELSEE

SEQ ID NO: 17 - protein, 379 aa, Vibrio phage nt-1
MNELYNNLMTLAESAEGKFFFADHLSPQGEKFRVFSYHIASYSDWLLPDALEARGIMFQLDENDEMIRIVSRPMEKFFNLGENPFTMDLDLTTTVQLMDKADGSLISTYLTGDNFALKSKTSIYSEQAVAANRYIKHVDNRDLWEFCDDCAAQNFTVNMEWCAPNNRIVLEYTEPKLIILNIRDNETGQYVSFDDIPIGALTRIKKWLVDEYDPMTAHVDDFVETLKAKKGIEGMILRLASGQSVKIKTTWYVDLHAQKDSVNSPKKLVTTILNKNHDDLYALFADDKPTIERIREFDDHVSKKVVESFHAVSQYYTKNRHLSRKDFAIAGQKALKPWEFGVAMIAYQNQTVEGVVTMLINAYLKRPELLIPEKYLSEV

SEQ ID NO: 18 - protein, 335 aa, Vibrio phage VH7D
MSFVKYTSLENSYRQAFVDKCDMLGVKEWVALEKIHGANFSFIVEFKPSTEEVPGEMSVTPAKRTSTIGANAMGDYDFYGCTSVVEAHIEKMQDISNWLFANDFIKNDETIIVYGELAGKGIQKEVNYGDKDFWAYDILCPETGEFLDWDVVLKACKFAGVKTTHEIARGTLDELLKIDPLFRSFHTPADVDSENVAEGFVVKQLKAEKRLHNGSRAILKVKNEKFKEKKNKQGKTPRAKVVLTEEQEKLHAAFSCYLTENRLRNVLSKIGKVEAKQFGMVSGLFVKDAKDEFERDERDEVAIPRDDWDVIKRSLVNVANEILRKNWLNIVDGTF

SEQ ID NO: 19 - protein, 339 aa, Klebsiella phage KP15
MFKKYSSLTNHYEGKFINGVIMNGLTGGVWVAREKIHGANFSFITDDGITVTPAKRTDVVKPAEDFYGCSAVVAKYSPGIRKMWETLKKTGTYDDLVIQVYGEFAGRGVQKDVDYGEKDFYVFDIRVNGEFLPDNLCSLISRSHGLKMAPLLGYGTFEEIKELPITFESVVNKANSGIGSDNTVYGEFVYPIMDVEEGNIAEGFVMKPVSPAFMPNGERVAIKCKTTKFTEKKAKKATRFNAPVSLSEKDKNQLDEFVCYLTENRVKNVLSKLDLASITAKDFGRIMGLTVQDAIEEISRNHGPFIEQFEDPAMAKKLFVTEAQNMIRPVWGKILNHEF

SEQ ID NO: 20 - protein, 335 aa, Escherichia phage JN02
MFKKYSSLENHYNSKFIEKLYTNGLTTGVWVAREKIHGTNFSLIIERDNVTCAKRTGPILPAEDFYGYEIVLKKYDKAIKAVQEVMESISTSVPVSYQVFGEFAGGGIQKGVDYGEKDFYVFDIIINTESDDTYYMSDYEMQDFCNTFGFKMAPMLGRGTFDSLIMIPNDLDSVLAAYNSTASEDLVEANNCVFDANVIGDNTAEGYVLKPCFPKWLSNGTRVAIKCKNSKFSEKKKSDKPVKTQVPLTEIDKNLLDVLACYVTLNRVNNVISKIGTVTPKDFGKVMGLTVQDILEETSREGIVLTSSDNPNLVKKELVRMVQDVLRPAWIELVS

SEQ ID NO: 21 - protein, 334 aa, Escherichia phage JS98
MFKKYSSLENHYNSKFIEKLRTNGLTGGEWVAREKIHGTNFSLIIERDAVTCAKRTGPILPAEDFYGYEIVLKNYADSIKSVQHLIESINYQSYQIYGELAGPGIQKNVDYGDKDFYVFDIRVTKEDGTESVLTDTLMEAFCIIHKFKVAPCLATGSFEDLIKLPNDFDSVIPDYNFAVDNAGLTIANSTDFIPKVEGKVFTAEGFVLKPDIPTWLPNGNRVAIKCKNSKFSEKKKSDKPIKAAVVLSQDDMDLMWQFTDYVTVNRINNVISKIGEVSKKDFGKVMGLTVQDILEEAAREELELTDAENPVEVKKQLVECVKDTLRAVWIELVS

SEQ ID NO: 22 - protein, 334 aa, Yersinia phage fPS-2
MFKKYSSLENHYNSKFIEKLYSLGLTGGEWVAREKIHGTNFSLIIERDKVTCAKRTGPILPAEDFFGYEIILKNYADSIKAVQDIMETSAVVSYQVFGEFAGPGIQKNVDYGDKDFYVFDIIVTTESGGVTYVDDYMMESFCNSFGFKIAPLLGRGKFEDLIKLPNDLDSVVQDYNFTVDHAGLVDANKCVWNAEAKGEVFTAEGYVLKPCYPSWLPNRNRVAIKCKNSKFSEKKKSDKPIKAKVELSEADNKLVGILACYVTLNRVNNVISKIGEIGPKDFGKVMGLTVQDILEETSREGITLTQADNPSLIKKELVKMVQDVLRPAWIELVS

SEQ ID NO: 23 - protein, 380 aa, Thermococcus barophilus
MVSLHFKHILLKLGLDKERIEILEMKGGIVEDEFEGLRYLRFKDSAKGLRRGTVVFNESDIILGFPHIKRVVHLRNGVKRIFKSKPFYVEEKVDGYNVRVAKVGEKILALTRGGFVCPFTTERIGDFINEQFFKDHPNLILCGEMAGPESPYLVEGPPYVEEDIQFFLFDIQEKRTGRSIPVEERIKLAEEYGIQSVEIFGLYSYEKIDELYELIERLSKEGREGVVMKSPDMKKIVKYVTPYANVNDIKIGSRIFFDLPHGYFMQRIKRLAFYIAEKRIRREDFDEYAKALGKALLQPFVESIWDVAAGEMIAEIFTVRVKKIETAYKMVSHFERMGLNIHIDDIEELGNGYWKITFKRVYDDATKEIRELWNGHAFVD

SEQ ID NO: 24 - protein, 335 aa, Vibrio phage ValKK3
MSFVKYTSLENSYRQAFVDKCDMLGVKEWVALEKIHGANFSFIVEFKPSTEQVPGEMSVTPAKRTSTIGANAMGDYDFYGCTSVVEAHIEKMQDISNWLFANDFIKNDETIIVYGELAGKGIQKEVNYGDKDFWAYDILCPETGEFLDWDVVLKACKFAGVKTTHEIARGTLDELLKIDPLFRSFHTPAAVDSENVAEGFVVKQLKAEKRLHNGSRAILKVKNEKFKEKKNKQGKTPRAKVVLTEEQEKLHAAFSCYLTENRLRNVLSKIGKVEAKQFGMVSGLFVKDAKDEFERDERDEVAIPRDDWDVIKRSLVNVANEILRKNWLNIVDGTF

SEQ ID NO: 25 - RNA, 91 nt, synthetic construct
  source 1..91: mol_type = other RNA; note = gRNA
nnnnnnnnnnnnnnngttttagagctagaaatagcaagttaaaataaggctagtccgttatcaacttgaaaaagtggcaccgagtcggtgc

SEQ ID NO: 26 - RNA, 96 nt, synthetic construct
  source 1..96: mol_type = other RNA; note = gRNA
nnnnnnnnnnnnnnnnnnnngttttagagctagaaatagcaagttaaaataaggctagtccgttatcaacttgaaaaagtggcaccgagtcggtgc

SEQ ID NO: 27 - RNA, 101 nt, synthetic construct
  source 1..101: mol_type = other RNA; note = gRNA
nnnnnnnnnnnnnnnnnnnnnnnnngttttagagctagaaatagcaagttaaaataaggctagtccgttatcaacttgaaaaagtggcaccgagtcggtgc

SEQ ID NO: 28 - RNA, 100 nt, synthetic construct
  source 1..100: mol_type = other RNA; note; note (original language) = 目标合成序列1
gactgatatacacaggccgatgtggttttagagctagaaatagcaagttaaaataaggctagtccgttatcaacttgaaaaagtggcaccgagtcggtgc

SEQ ID NO: 29 - RNA, 24 nt, synthetic construct
  source 1..24: mol_type = other RNA; note = g1
gactgatatacacaggccgatgtg

SEQ ID NO: 30 - RNA, 36 nt, synthetic construct
  source 1..36: mol_type = other RNA; note = g2
gttttagagctagaaatagcaagttaaaataaggct

SEQ ID NO: 31 - RNA, 40 nt, synthetic construct
  source 1..40: mol_type = other RNA; note = g3
agtccgttatcaacttgaaaaagtggcaccgagtcggtgc

SEQ ID NO: 32 - RNA, 50 nt, synthetic construct
  source 1..50: mol_type = other RNA; note = g4
gactgatatacacaggccgatgtggttttagagctagaaatagcaagtta

SEQ ID NO: 33 - RNA, 50 nt, synthetic construct
  source 1..50: mol_type = other RNA; note = g5
aaataaggctagtccgttatcaacttgaaaaagtggcaccgagtcggtgc

SEQ ID NO: 34 - RNA, 41 nt, synthetic construct
  source 1..41: mol_type = other RNA; note; note (original language) = 底物序列
nnnnnnnnnnnnnnngttttagagctagaaatagcaagtta

SEQ ID NO: 35 - RNA, 51 nt, synthetic construct
  source 1..51: mol_type = other RNA; note; note (original language) = 底物序列
nnnnnnnnnnnnnnnnnnnnnnnnngttttagagctagaaatagcaagtta

SEQ ID NO: 36 - RNA, 26 nt, synthetic construct
  source 1..26: mol_type = other RNA; note; note (original language) = 底物序列
gttttagagctagaaatagcaagtta

SEQ ID NO: 37 - DNA, 60 bp, synthetic construct
  source 1..60: mol_type = other DNA; note = g-D
tgataacggactagccttattttaacttgctatttctagctctaaaaccacatcggcctg

SEQ ID NO: 38 - RNA, 36 nt, synthetic construct; identical to SEQ ID NO: 30
  source 1..36: mol_type = other RNA; note = P-g2

SEQ ID NO: 39 - DNA, 51 bp, synthetic construct
  source 1..51: mol_type = other DNA; note; note (original language) = 模板核酸链
tgataacggactagccttattttaacttgctatttctagctctaaaacnnn

SEQ ID NO: 40 - DNA, 73 bp, synthetic construct
  source 1..73: mol_type = other DNA; note; note (original language) = 模板核酸链
tgataacggactagccttattttaacttgctatttctagctctaaaacnnnnnnnnnnnnnnnnnnnnnnnnn

SEQ ID NO: 41 - RNA, 142 nt, synthetic construct
  source 1..142: mol_type = other RNA; note; note (original language) = 目标合成序列2
tgatatacacaggccgatgtggttgtagctccctttctcatttcggaaacgaaatgagaaccgttgctacaataaggccgtctgaaaagatgtgccgcaacgctctgccccttaaagcctctgctttaaggggcatcgtttc

SEQ ID NO: 42 - RNA, 136 nt, synthetic construct
  source 1..136: mol_type = other RNA; note = gRNA
nnnnnnnnnnnnnnngttgtagctccctttctcatttcggaaacgaaatgagaaccgttgctacaataaggccgtctgaaaagatgtgccgcaacgctctgccccttaaagcctctgctttaaggggcatcgtttc

SEQ ID NO: 43 - RNA, 146 nt, synthetic construct
  source 1..146: mol_type = other RNA; note = gRNA
nnnnnnnnnnnnnnnnnnnnnnnnngttgtagctccctttctcatttcggaaacgaaatgagaaccgttgctacaataaggccgtctgaaaagatgtgccgcaacgctctgccccttaaagcctctgctttaaggggcatcgtttc

SEQ ID NO: 44 - RNA, 39 nt, synthetic construct
  source 1..39: mol_type = other RNA; note = Ng1
tgatatacacaggccgatgtggttgtagctccctttctc

SEQ ID NO: 45 - RNA, 45 nt, synthetic construct
  source 1..45: mol_type = other RNA; note = Ng2
atttcggaaacgaaatgagaaccgttgctacaataaggccgtctg

SEQ ID NO: 46 - RNA, 58 nt, synthetic construct
  source 1..58: mol_type = other RNA; note = Ng3
aaaagatgtgccgcaacgctctgccccttaaagcctctgctttaaggggcatcgtttc

SEQ ID NO: 47 - RNA, 18 nt, synthetic construct
  source 1..18: mol_type = other RNA; note; note (original language) = 底物序列
gttgtagctccctttctc

SEQ ID NO: 48 - RNA, 71 nt, synthetic construct
  source 1..71: mol_type = other RNA; note = Ng4
tgatatacacaggccgatgtggttgtagctccctttctcatttcggaaacgaaatgagaaccgttgctaca

SEQ ID NO: 49 - RNA, 71 nt, synthetic construct
  source 1..71: mol_type = other RNA; note = Ng5
ataaggccgtctgaaaagatgtgccgcaacgctctgccccttaaagcctctgctttaaggggcatcgtttc

SEQ ID NO: 50 - RNA, 50 nt, synthetic construct
  source 1..50: mol_type = other RNA; note; note (original language) = 底物序列
gttgtagctccctttctcatttcggaaacgaaatgagaaccgttgctaca

SEQ ID NO: 51 - DNA, 69 bp, synthetic construct
  source 1..69: mol_type = other DNA; note = Ng-D
ggcacatcttttcagacggccttattgtagcaacggttctcatttcgtttccgaaatgagaaagggagc

SEQ ID NO: 52 - RNA, 45 nt, synthetic construct; identical to SEQ ID NO: 45
  source 1..45: mol_type = other RNA; note = P-Ng2